European Patent Application EP 4 299 748 A1, published January 3, 2024. Title: Method for manufacturing alfalfa mosaic virus-like particles using plant expression system and application thereof. Applicant: BioApplications Inc. The sequence listing filed with the application follows.

SEQUENCE LISTING (11 sequences)

SEQ ID NO: 1 - DNA, 231 bp, Artificial Sequence
  DNA sequence of RuBisCO transit peptide
atggcttcctctatgctctcttccgctactatggttgcctctccggctcaggccactatggtcgctcctttcaacggacttaagtcctccgctgccttcccagccacccgcaaggctaacaacgacactacttccatcacaagcaacggcggaagagttaactgcatgcaggtgtggcctccgattggaaagaagaagtttgagactctctcttaccttcctgaccttacc

SEQ ID NO: 2 - protein, 23 aa, Artificial Sequence
  Amino acid sequence of RuBisCO transit peptide
CMQVWPPIGKKKFETLSYLPDLT

SEQ ID NO: 3 - DNA, 663 bp, Artificial Sequence
  Optimized DNA sequence of Alfalfa mosaic virus capsid
atgagttcttcacaaaagaaagctggtggtaaagctggtaagcctactaagagatctcagaactatgctgccttacggaaagctcagcttccgaaaccaccggccttgaaggtcccagtggtaaagccaacaaatacaatactgccacagactggttgcgtttggcaatcgttagggacgcctttgagtctttcatcttttaatggattaggtgttagattcctttatagttttcttaaggactttgcaggaccaagaatcctcgaagaagatctgatttacaggatggtgttttccattacacccagctacgctggcaccttttgtcttactgatgacgtgaccactgaagatggtagggcagttgctcatggaaatcctatgcaagaattccctcacggcgcatttcacgctaatgaaaagtttgggtttgagttggtttttacagctcctacccatgctggaatgcaaaaccaaaatttcaagcattcctatgccgttgcgttgtgtttggattttgacgcacagcctgagggatctaaaaatccttcatataggttcaacgaggtctgggttgagagaaaagcattcccacgagcaggacccctacgctctttgattactgtaggactactcgatgaagctgatgatcttgatcgtcat

SEQ ID NO: 4 - protein, 221 aa, Artificial Sequence
  Amino acid sequence of Alfalfa mosaic virus capsid
MSSSQKKAGGKAGKPTKRSQNYAALRKAQLPKPPALKVPVVKPTNTILPQTGCVWQSLGTPLSLSSFNGLGVRFLYSFLKDFAGPRILEEDLIYRMVFSITPSYAGTFCLTDDVTTEDGRAVAHGNPMQEFPHGAFHANEKFGFELVFTAPTHAGMQNQNFKHSYAVALCLDFDAQPEGSKNPSYRFNEVWVERKAFPRAGPLRSLITVGLLDEADDLDRH

SEQ ID NO: 5 - DNA, 18 bp, Artificial Sequence
  DNA sequence of polyhistidine-tag
caccaccatcaccaccat

SEQ ID NO: 6 - protein, 6 aa, Artificial Sequence
  Amino acid sequence of polyhistidine-tag
HHHHHH

SEQ ID NO: 7 - DNA, 12 bp, Artificial Sequence
  DNA sequence of HDEL
ctctagctcgag

SEQ ID NO: 8 - protein, 4 aa, Artificial Sequence
  Amino acid sequence of HDEL
HDEL

SEQ ID NO: 9 - DNA, 251 bp, Artificial Sequence
  DNA sequence of New BiP signal peptide
atggctcgctcgtttggagctaacagtaccgttgtgttggcgatcatcttcttcggtgagtgattttccgatcttcttctccgatttagatctcctctacattgttgcttaatctcagaaccttttttcgttgttcctggatctgaatgtgtttgtttgcaatttcacgatcttaaaaggttagatctcgattggtattgacgattggaatctttacgatttcaggatgtttatttgcgttgtcctctgca

SEQ ID NO: 10 - DNA, 666 bp, Artificial Sequence
  DNA sequence of Alfalfa mosaic virus capsid
atgagttcttcacaaaagaaagctggtgggaaagctggtaaacctactaaacgttctcagaactatgctgccttacgcaaagctcaactgccgaagcctccggcgttgaaagtcccggttgtaaaaccgacgaatactatactgccacagacgggctgcgtgtggcaaagcctcgggacccctctgagtctgagctcttttaatgggctcggcgtgagattcctctacagttttctgaaggatttcgcgggacctcggatcctcgaagaggatctgatttacaggatggtgttttccataacaccgtcctatgccggcaccttttgtctcactgatgacgtgacgactgaggatggtagggccgttgcgcatggtaatcccatgcaagaatttcctcatggcgcgtttcacgctaatgagaagttcgggtttgagttggtcttcacagctcctacccatgcgggaatgcaaaaccaaaatttcaagcattcctatgccgtagccctctgtctggacttcgacgcgcagcctgagggatctaaaaatccctcataccgattcaacgaagtttgggtcgagagaaaggcgttcccgcgagcagggcccctccgcagtttgattactgtggggctgctcgacgaagctgacgatcttgatcgtcattga

SEQ ID NO: 11 - DNA, 971 bp, Artificial Sequence
  Full insert seuqence(NR-AMV-His tag)
tctagaattattacatcaaaacaaaaaatggcttcctctatgctctcttccgctactatggttgcctctccggctcaggccactatggtcgctcctttcaacggacttaagtcctccgctgccttcccagccacccgcaaggctaacaacgacactacttccatcacaagcaacggcggaagagttaactgcatgcaggtgtggcctccgattggaaagaagaagtttgagactctctcttaccttcctgaccttaccggatccatgagttcttcacaaaagaaagctggtggtaaagctggtaagcctactaagagatctcagaactatgctgccttacggaaagctcagcttccgaaaccaccggccttgaaggtcccagtggtaaagccaacaaatacaatactgccacagactggttgcgtttggcaatcgttagggacgcctttgagtctttcatcttttaatggattaggtgttagattcctttatagttttcttaaggactttgcaggaccaagaatcctcgaagaagatctgatttacaggatggtgttttccattacacccagctacgctggcaccttttgtcttactgatgacgtgaccactgaagatggtagggcagttgctcatggaaatcctatgcaagaattccctcacggcgcatttcacgctaatgaaaagtttgggtttgagttggtttttacagctcctacccatgctggaatgcaaaaccaaaatttcaagcattcctatgccgttgcgttgtgtttggattttgacgcacagcctgagggatctaaaaatccttcatataggttcaacgaggtctgggttgagagaaaagcattcccacgagcaggacccctacgctctttgattactgtaggactactcgatgaagctgatgatcttgatcgtcatccccggggtcaccaccatcaccaccattagagctctaactcgag